European Patent Application EP 4 467 651 A1, published November 27, 2024. Title: Method for regulating and controlling heterologous synthetic flavonoid compound and use thereof. Applicant: CAS CENTER FOR EXCELLENCE IN MOLECULAR PLANT SCIENCES. Application WO PCT/CN2023/073308, filed January 20, 2023. The sequence listing filed with the application follows.

SEQUENCE LISTING (17 sequences)

SEQ ID NO: 1 - DNA, 85 bp, synthetic construct
  source 1..85: mol_type = other DNA
tttctgttgggccattgcattgccactgattttccaacatataaaaagacaagcccgaacagtcgtccgggctttttttctcgag

SEQ ID NO: 2 - DNA, 109 bp, synthetic construct
  source 1..109: mol_type = other DNA
gttttcgaagctggtgtcgttcattttctgttgggccattgcattgccactgattttccaacatataaaaagacaagcccgaacagtcgtccgggctttttttctcgag

SEQ ID NO: 3 - DNA, 109 bp, synthetic construct
  source 1..109: mol_type = other DNA
gaaaataatgacttgctggctcattttctgttgggccattgcattgccactgattttccaacatataaaaagacaagcccgaacagtcgtccgggctttttttctcgag

SEQ ID NO: 4 - DNA, 109 bp, synthetic construct
  source 1..109: mol_type = other DNA
tttttcgtataacgtcttagccattttctgttgggccattgcattgccactgattttccaacatataaaaagacaagcccgaacagtcgtccgggctttttttctcgag

SEQ ID NO: 5 - DNA, 109 bp, synthetic construct
  source 1..109: mol_type = other DNA
gtgtttgataaatttctctgccattttctgttgggccattgcattgccactgattttccaacatataaaaagacaagcccgaacagtcgtccgggctttttttctcgag

SEQ ID NO: 6 - DNA, 109 bp, synthetic construct
  source 1..109: mol_type = other DNA
tatggcaatatacgccactgtcattttctgttgggccattgcattgccactgattttccaacatataaaaagacaagcccgaacagtcgtccgggctttttttctcgag

SEQ ID NO: 7 - DNA, 109 bp, synthetic construct
  source 1..109: mol_type = other DNA
ggcaagctctttacgtgaggacattttctgttgggccattgcattgccactgattttccaacatataaaaagacaagcccgaacagtcgtccgggctttttttctcgag

SEQ ID NO: 8 - DNA, 109 bp, synthetic construct
  source 1..109: mol_type = other DNA
gccagtaatcactgcacgtttcattttctgttgggccattgcattgccactgattttccaacatataaaaagacaagcccgaacagtcgtccgggctttttttctcgag

SEQ ID NO: 9 - DNA, 109 bp, synthetic construct
  source 1..109: mol_type = other DNA
ggcaataacaattttatccagcattttctgttgggccattgcattgccactgattttccaacatataaaaagacaagcccgaacagtcgtccgggctttttttctcgag

SEQ ID NO: 10 - DNA, 108 bp, synthetic construct
  source 1..108: mol_type = other DNA
ttttttaatcttacgaatatccattttctgttgggccattgcattgccactgattttccaacatataaaaagacaagcccgaacagtcgccgggctttttttctcgag

SEQ ID NO: 11 - DNA, 109 bp, synthetic construct
  source 1..109: mol_type = other DNA
atacaactcagcttgcttttgcattttctgttgggccattgcattgccactgattttccaacatataaaaagacaagcccgaacagtcgtccgggctttttttctcgag

SEQ ID NO: 12 - DNA, 109 bp, synthetic construct
  source 1..109: mol_type = other DNA
tttctgatatagcggattagccattttctgttgggccattgcattgccactgattttccaacatataaaaagacaagcccgaacagtcgtccgggctttttttctcgag

SEQ ID NO: 13 - DNA, 109 bp, synthetic construct
  source 1..109: mol_type = other DNA
aatgttcatttcacgctttaacattttctgttgggccattgcattgccactgattttccaacatataaaaagacaagcccgaacagtcgtccgggctttttttctcgag

SEQ ID NO: 14 - protein, 36 aa, synthetic construct
KAKLKEEEERKQREEEERIKRLEELAKRKEEERKGT

SEQ ID NO: 15 - protein, 7 aa, synthetic construct
GVKESLV

SEQ ID NO: 16 - protein, 57 aa, synthetic construct
AEYVRALFDFNGNDEEDLPFKKGDILRIRDKPEEQWWNAEDSEGKRGMIPVPYVEKY

SEQ ID NO: 17 - protein, 11 aa, synthetic construct
PPPALPPKRRR